European Patent Application EP 4 328 308 A1, published February 28, 2024. Title: Modified tRNA Synthetase for [...]. Applicant: Technische Universitaet Berlin. Application EP. The sequence listing filed with the application follows.

SEQUENCE LISTING (11 sequences)

SEQ ID NO: 1 - protein, 416 aa, Methanococcoides burtonii
  VARIANT 346: note = X(346) -> F
  VARIANT 308: note = X2(308) -> N, Q, L, M, G, A
  VARIANT 310: note = X3(310) -> C, G, W, A
  VARIANT 379: note = X4(379) -> S, T, W
MEKQLLDVLVELNGVWLSRSGLLHGIRNFEITTKHIHIETDCGARFTVRNSRSSRSARSLRHNKYRKPCKRCRPADEQIDRFVKKTFKEKRQTVSVFSSPKKHVPKKPKVAVIKSFSISTPSPKEASVSNSIPTPSISVVKDEVKVPEVKYTPSQIERLKTLMSPDDKIPIQDELPEFKVLEKELIQRRRDDLKKMYEEDREDRLGKLERDITEFFVDRGFLEIKSPIMIPFEYIERMGIDKDDHLNKQIFRVDESMCLRPMLAPCLYNYLRKLDKVLPDPIRIFEIGPCYRKESDGSSHLEEFTMVXFXQMGSGCTRENMEALIDEFLEHLGIEYEIEADNCMVXGDTIDIMHGDLELSSAVVGPIPLDREWGVNKPXMGAGFGLERLLKVRHNYTNIRRASRSELYYNGINTNL

SEQ ID NO: 2 - RNA, 72 nt, synthetic construct
  source 1..72: mol_type = other RNA
ggagacttgatcatgtagatcgaacggactctaaatccgttcagccgggttagattcccggagtttccgcca

SEQ ID NO: 3 - protein, 416 aa, synthetic construct
MEKQLLDVLVELNGVWLSRSGLLHGIRNFEITTKHIHIETDCGARFTVRNSRSSRSARSLRHNKYRKPCKRCRPADEQIDRFVKKTFKEKRQTVSVFSSPKKHVPKKPKVAVIKSFSISTPSPKEASVSNSIPTPSISVVKDEVKVPEVKYTPSQIERLKTLMSPDDKIPIQDELPEFKVLEKELIQRRRDDLKKMYEEDREDRLGKLERDITEFFVDRGFLEIKSPIMIPFEYIERMGIDKDDHLNKQIFRVDESMCLRPMLAPCLYNYLRKLDKVLPDPIRIFEIGPCYRKESDGSSHLEEFTMVNFCQMGSGCTRENMEALIDEFLEHLGIEYEIEADNCMVFGDTIDIMHGDLELSSAVVGPIPLDREWGVNKPWMGAGFGLERLLKVRHNYTNIRRASRSELYYNGINTNL

SEQ ID NO: 4 - protein, 416 aa, synthetic construct
MEKQLLDVLVELNGVWLSRSGLLHGIRNFEITTKHIHIETDCGARFTVRNSRSSRSARSLRHNKYRKPCKRCRPADEQIDRFVKKTFKEKRQTVSVFSSPKKHVPKKPKVAVIKSFSISTPSPKEASVSNSIPTPSISVVKDEVKVPEVKYTPSQIERLKTLMSPDDKIPIQDELPEFKVLEKELIQRRRDDLKKMYEEDREDRLGKLERDITEFFVDRGFLEIKSPIMIPFEYIERMGIDKDDHLNKQIFRVDESMCLRPMLAPCLYNYLRKLDKVLPDPIRIFEIGPCYRKESDGSSHLEEFTMVAFAQMGSGCTRENMEALIDEFLEHLGIEYEIEADNCMVFGDTIDIMHGDLELSSAVVGPIPLDREWGVNKPWMGAGFGLERLLKVRHNYTNIRRASRSELYYNGINTNL

SEQ ID NO: 5 - protein, 416 aa, synthetic construct
MEKQLLDVLVELNGVWLSRSGLLHGIRNFEITTKHIHIETDCGARFTVRNSRSSRSARSLRHNKYRKPCKRCRPADEQIDRFVKKTFKEKRQTVSVFSSPKKHVPKKPKVAVIKSFSISTPSPKEASVSNSIPTPSISVVKDEVKVPEVKYTPSQIERLKTLMSPDDKIPIQDELPEFKVLEKELIQRRRDDLKKMYEEDREDRLGKLERDITEFFVDRGFLEIKSPIMIPFEYIERMGIDKDDHLNKQIFRVDESMCLRPMLAPCLYNYLRKLDKVLPDPIRIFEIGPCYRKESDGSSHLEEFTMVGFGQMGSGCTRENMEALIDEFLEHLGIEYEIEADNCMVFGDTIDIMHGDLELSSAVVGPIPLDREWGVNKPWMGAGFGLERLLKVRHNYTNIRRASRSELYYNGINTNL

SEQ ID NO: 6 - protein, 416 aa, synthetic construct
MEKQLLDVLVELNGVWLSRSGLLHGIRNFEITTKHIHIETDCGARFTVRNSRSSRSARSLRHNKYRKPCKRCRPADEQIDRFVKKTFKEKRQTVSVFSSPKKHVPKKPKVAVIKSFSISTPSPKEASVSNSIPTPSISVVKDEVKVPEVKYTPSQIERLKTLMSPDDKIPIQDELPEFKVLEKELIQRRRDDLKKMYEEDREDRLGKLERDITEFFVDRGFLEIKSPIMIPFEYIERMGIDKDDHLNKQIFRVDESMCLRPMLAPCLYNYLRKLDKVLPDPIRIFEIGPCYRKESDGSSHLEEFTMVMFWQMGSGCTRENMEALIDEFLEHLGIEYEIEADNCMVFGDTIDIMHGDLELSSAVVGPIPLDREWGVNKPWMGAGFGLERLLKVRHNYTNIRRASRSELYYNGINTNL

SEQ ID NO: 7 - protein, 416 aa, synthetic construct
MEKQLLDVLVELNGVWLSRSGLLHGIRNFEITTKHIHIETDCGARFTVRNSRSSRSARSLRHNKYRKPCKRCRPADEQIDRFVKKTFKEKRQTVSVFSSPKKHVPKKPKVAVIKSFSISTPSPKEASVSNSIPTPSISVVKDEVKVPEVKYTPSQIERLKTLMSPDDKIPIQDELPEFKVLEKELIQRRRDDLKKMYEEDREDRLGKLERDITEFFVDRGFLEIKSPIMIPFEYIERMGIDKDDHLNKQIFRVDESMCLRPMLAPCLYNYLRKLDKVLPDPIRIFEIGPCYRKESDGSSHLEEFTMVQFWQMGSGCTRENMEALIDEFLEHLGIEYEIEADNCMVFGDTIDIMHGDLELSSAVVGPIPLDREWGVNKPWMGAGFGLERLLKVRHNYTNIRRASRSELYYNGINTNL

SEQ ID NO: 8 - protein, 416 aa, synthetic construct
MEKQLLDVLVELNGVWLSRSGLLHGIRNFEITTKHIHIETDCGARFTVRNSRSSRSARSLRHNKYRKPCKRCRPADEQIDRFVKKTFKEKRQTVSVFSSPKKHVPKKPKVAVIKSFSISTPSPKEASVSNSIPTPSISVVKDEVKVPEVKYTPSQIERLKTLMSPDDKIPIQDELPEFKVLEKELIQRRRDDLKKMYEEDREDRLGKLERDITEFFVDRGFLEIKSPIMIPFEYIERMGIDKDDHLNKQIFRVDESMCLRPMLAPCLYNYLRKLDKVLPDPIRIFEIGPCYRKESDGSSHLEEFTMVLFWQMGSGCTRENMEALIDEFLEHLGIEYEIEADNCMVFGDTIDIMHGDLELSSAVVGPIPLDREWGVNKPWMGAGFGLERLLKVRHNYTNIRRASRSELYYNGINTNL

SEQ ID NO: 9 - protein, 416 aa, synthetic construct
MEKQLLDVLVELNGVWLSRSGLLHGIRNFEITTKHIHIETDCGARFTVRNSRSSRSARSLRHNKYRKPCKRCRPADEQIDRFVKKTFKEKRQTVSVFSSPKKHVPKKPKVAVIKSFSISTPSPKEASVSNSIPTPSISVVKDEVKVPEVKYTPSQIERLKTLMSPDDKIPIQDELPEFKVLEKELIQRRRDDLKKMYEEDREDRLGKLERDITEFFVDRGFLEIKSPIMIPFEYIERMGIDKDDHLNKQIFRVDESMCLRPMLAPCLYNYLRKLDKVLPDPIRIFEIGPCYRKESDGSSHLEEFTMVNFWQMGSGCTRENMEALIDEFLEHLGIEYEIEADNCMVFGDTIDIMHGDLELSSAVVGPIPLDREWGVNKPTMGAGFGLERLLKVRHNYTNIRRASRSELYYNGINTNL

SEQ ID NO: 10 - DNA, 1251 bp, synthetic construct
  source 1..1251: mol_type = other DNA
atggaaaagcagctcctggacgtgctggtggaactgaatggcgtgtggctgagcagatctggcctgctgcacggcatccggaacttcgagatcaccaccaagcacatccacatcgagacagactgcggcgccagattcaccgtgcggaacagcagatctagcagaagcgccagaagcctgcggcacaacaagtacagaaagccctgcaagagatgcagacccgccgacgagcagatcgacagattcgtgaagaaaaccttcaaagaaaagcggcagaccgtgtccgtgttcagcagccccaagaaacacgtgcccaaaaagcccaaggtggccgtgatcaagagcttcagcatcagcaccccatctccaaaagaggccagcgtcagcaacagcatccctacacctagcatcagcgtggtcaaggacgaagtgaaggtgccagaagtgaagtacacccctagccagatcgagcggctgaaaaccctgatgagccccgacgacaagatccccatccaggatgagctgcccgagttcaaggtgctggaaaaagagctgatccagcggcggagggacgacctgaagaagatgtacgaagaggacagagaggaccggctgggcaagctggaaagagacatcaccgagttcttcgtggaccggggcttcctggaaatcaagagccccatcatgatcccgttcgagtacatcgagcggatgggcatcgacaaggacgaccacctgaacaagcagattttcagagtggacgagagcatgtgcctgcggcctatgctggccccttgcctgtacaactacctgcggaagctggataaggtgctgcccgatcctatccgcatctttgagatcggcccctgctaccggaaagagagcgacggatctagccacctggaagagttcaccatggtcaatttctggcagatgggcagcggctgcacccgcgagaatatggaagccctgatcgacgagttcctggaacacctgggaatcgagtacgagatcgaggccgacaactgcatggtgttcggcgacaccatcgacatcatgcacggcgacctggaactgtctagcgccgttgtgggacccattcctctggatagagaatggggcgtgaacaagcccacaatgggagccggctttggcctggaaagactgctgaaagtgcgccacaactacaccaacatcagacgggccagccgcagcgagctgtactacaacggcatcaacaccaacctgtga

SEQ ID NO: 11 - DNA, 51 bp, synthetic construct
  source 1..51: mol_type = other DNA
gcttgtcctgttcctctgcagctgcctcctctggaaagactgaccctggat